European Patent Specification EP 3 472 199 B1, published November 1, 2023. Title: Peptide and antibodies for use in diagnosis. Applicant: Skiöldebrand Eva Lindahl Anders Ekman Stina. The sequence listing filed with the application follows.

SEQUENCE LISTING (6 sequences)

SEQ ID NO: 1 - protein, 5 aa, Equus caballus
SGPTH

SEQ ID NO: 2 - protein, 9 aa, Artificial Sequence
  Peptide used for immunisation
SGPTHGGGC

SEQ ID NO: 3 - protein, 9 aa, Equus caballus
SGPTHEGVC

SEQ ID NO: 4 - protein, 15 aa, Equus caballus
PPGYSGPTHEGVGMC

SEQ ID NO: 5 - protein, 11 aa, Equus caballus
SGPTHEGVGMA

SEQ ID NO: 6 - protein, 11 aa, Homo sapiens
SGPTHQGVGLA